European Patent Specification EP 4 590 851 B1, published September 2, 2026. Title: Padlock Blocking Oligonucleotide. Applicant: Bo Xu. Application WO. The sequence listing filed with the application follows.

SEQUENCE LISTING (11 sequences)

SEQ ID NO: 1 - DNA, 69 bp, synthetic construct
  source 1..69: mol_type = other DNA; note = Padlock
ctcacccaactacatacaccaacacaaatccgcgtgataacgaaccacacacacacaacaacaccacca

SEQ ID NO: 2 - DNA, 50 bp, synthetic construct
  source 1..50: mol_type = other DNA; note = Ligation template
actcccactccactgggtctggtcaaaaagttgggtgagtggtggtgttg

SEQ ID NO: 3 - DNA, 38 bp, synthetic construct
  source 1..38: mol_type = other DNA; note = Blocking oligo 13+13
gtagttgggtgagccgataacactttggtggtgttgtt

SEQ ID NO: 4 - DNA, 50 bp, synthetic construct
  source 1..50: mol_type = other DNA; note = Blocking oligo 19+19
gtgtatgtagttgggtgagccgataacactttggtggtgttgttgtgttg

SEQ ID NO: 5 - DNA, 46 bp, synthetic construct
  source 1..46: mol_type = other DNA; note = Blocking oligo 17+17
gtatgtagttgggtgagccgataacactttggtggtgttgttgtgt

SEQ ID NO: 6 - DNA, 42 bp, synthetic construct
  source 1..42: mol_type = other DNA; note = Blocking oligo 15+15
atgtagttgggtgagccgataacactttggtggtgttgttgt

SEQ ID NO: 7 - DNA, 30 bp, synthetic construct
  source 1..30: mol_type = other DNA; note = Conjugation oligo1 for padlock hybridization
tggttcgttatcacgcggatttgtaaaaaa

SEQ ID NO: 8 - DNA, 33 bp, synthetic construct
  source 1..33: mol_type = other DNA; note = Conjugation oligo2 For ligation template hybridization
aaaaaattgaccagacccagtggagtgggagtc

SEQ ID NO: 9 - DNA, 15 bp, synthetic construct
  source 1..15: mol_type = other DNA; note = Detection oligo
tacatacaccaacac

SEQ ID NO: 10 - DNA, 22 bp, synthetic construct
  source 1..22: mol_type = other DNA; note = Key oligo short 22nt
caccaaagtgttatcggctcaa

SEQ ID NO: 11 - DNA, 34 bp, synthetic construct
  source 1..34: mol_type = other DNA; note = Key oligo long 34nt
caacaacaccaaagtgttatcggctcaaactaca